European Patent Application EP 4 722 255 A1, published April 8, 2026. Title: 嵌合抗原受体及其用途. Applicant: 深圳普瑞金生物药业股份有限公司. Application CN. The sequence listing filed with the application follows.

SEQUENCE LISTING (24 sequences)

SEQ ID NO: 1 - protein, 21 aa, synthetic construct
MALPVTALLLPLALLLHAARP

SEQ ID NO: 2 - protein, 5 aa, synthetic construct
TYFMA

SEQ ID NO: 3 - protein, 17 aa, synthetic construct
GGIRWSDGVPHYADSVK

SEQ ID NO: 4 - protein, 13 aa, synthetic construct
ASRGIADGSDFGS

SEQ ID NO: 5 - protein, 113 aa, synthetic construct
RVKFSRSADAPAYQQGQNQLYNELNLGRREEYDVLDKRRGRDPEMGGKPQRRKNPQEGLYNELQKDKMAEAYSEIGMKGERRRGKGHDGLYQGLSTATKDTYDALHMQALPPR

SEQ ID NO: 6 - protein, 18 aa, synthetic construct
EGRGSLLTCGDVEENPGP

SEQ ID NO: 7 - protein, 161 aa, synthetic construct
RISKPHLRSISIQCYLCLLLNSHFLTEAGIHVFILGCFSAGLPKTEANWVNVISDLKKIEDLIQSMHIDATLYTESDVHPSCKVTAMKCFLLELQVISLESGDASIHDTVENLIILANNSLSSNGNVTESGCKECEELEEKNIKEFLQSFVHIVQMFINTS

SEQ ID NO: 8 - protein, 120 aa, synthetic construct
EVQLQASGGGLAQPGGSLRLSCAASGRTFSTYFMAWFRQPPGKGLEYVGGIRWSDGVPHYADSVKGRFTISRDNAKNTVYLQMNSLRAEDTAVYFCASRGIADGSDFGSYGQGTQVTVSS

SEQ ID NO: 9 - protein, 107 aa, synthetic construct
IEVMYPPPYLDNEKSNGTIIHVKGKHLCPSPLFPGPSKPFWVLVVVGGVLACYSLLVTVAFIIFWVRSKRSRLLHSDYMNMTPRRPGPTRKHYQPYAPPRDFAAYRS

SEQ ID NO: 10 - protein, 220 aa, synthetic construct
IEVMYPPPYLDNEKSNGTIIHVKGKHLCPSPLFPGPSKPFWVLVVVGGVLACYSLLVTVAFIIFWVRSKRSRLLHSDYMNMTPRRPGPTRKHYQPYAPPRDFAAYRSRVKFSRSADAPAYQQGQNQLYNELNLGRREEYDVLDKRRGRDPEMGGKPQRRKNPQEGLYNELQKDKMAEAYSEIGMKGERRRGKGHDGLYQGLSTATKDTYDALHMQALPPR

SEQ ID NO: 11 - protein, 340 aa, synthetic construct
EVQLQASGGGLAQPGGSLRLSCAASGRTFSTYFMAWFRQPPGKGLEYVGGIRWSDGVPHYADSVKGRFTISRDNAKNTVYLQMNSLRAEDTAVYFCASRGIADGSDFGSYGQGTQVTVSSIEVMYPPPYLDNEKSNGTIIHVKGKHLCPSPLFPGPSKPFWVLVVVGGVLACYSLLVTVAFIIFWVRSKRSRLLHSDYMNMTPRRPGPTRKHYQPYAPPRDFAAYRSRVKFSRSADAPAYQQGQNQLYNELNLGRREEYDVLDKRRGRDPEMGGKPQRRKNPQEGLYNELQKDKMAEAYSEIGMKGERRRGKGHDGLYQGLSTATKDTYDALHMQALPPR

SEQ ID NO: 12 - protein, 361 aa, synthetic construct
MALPVTALLLPLALLLHAARPEVQLQASGGGLAQPGGSLRLSCAASGRTFSTYFMAWFRQPPGKGLEYVGGIRWSDGVPHYADSVKGRFTISRDNAKNTVYLQMNSLRAEDTAVYFCASRGIADGSDFGSYGQGTQVTVSSIEVMYPPPYLDNEKSNGTIIHVKGKHLCPSPLFPGPSKPFWVLVVVGGVLACYSLLVTVAFIIFWVRSKRSRLLHSDYMNMTPRRPGPTRKHYQPYAPPRDFAAYRSRVKFSRSADAPAYQQGQNQLYNELNLGRREEYDVLDKRRGRDPEMGGKPQRRKNPQEGLYNELQKDKMAEAYSEIGMKGERRRGKGHDGLYQGLSTATKDTYDALHMQALPPR

SEQ ID NO: 13 - protein, 540 aa, synthetic construct
MALPVTALLLPLALLLHAARPEVQLQASGGGLAQPGGSLRLSCAASGRTFSTYFMAWFRQPPGKGLEYVGGIRWSDGVPHYADSVKGRFTISRDNAKNTVYLQMNSLRAEDTAVYFCASRGIADGSDFGSYGQGTQVTVSSIEVMYPPPYLDNEKSNGTIIHVKGKHLCPSPLFPGPSKPFWVLVVVGGVLACYSLLVTVAFIIFWVRSKRSRLLHSDYMNMTPRRPGPTRKHYQPYAPPRDFAAYRSRVKFSRSADAPAYQQGQNQLYNELNLGRREEYDVLDKRRGRDPEMGGKPQRRKNPQEGLYNELQKDKMAEAYSEIGMKGERRRGKGHDGLYQGLSTATKDTYDALHMQALPPREGRGSLLTCGDVEENPGPRISKPHLRSISIQCYLCLLLNSHFLTEAGIHVFILGCFSAGLPKTEANWVNVISDLKKIEDLIQSMHIDATLYTESDVHPSCKVTAMKCFLLELQVISLESGDASIHDTVENLIILANNSLSSNGNVTESGCKECEELEEKNIKEFLQSFVHIVQMFINTS

SEQ ID NO: 14 - protein, 518 aa, synthetic construct
MALPVTALLLPLALLLHAARPEVQLQASGGGLAQPGGSLRLSCAASGRTFSTYFMAWFRQPPGKGLEYVGGIRWSDGVPHYADSVKGRFTISRDNAKNTVYLQMNSLRAEDTAVYFCASRGIADGSDFGSYGQGTQVTVSSEPKSCDKTHTCPPCPKPFWVLVVVGGVLACYSLLVTVAFIIFWVRSKRSRLLHSDYMNMTPRRPGPTRKHYQPYAPPRDFAAYRSRVKFSRSADAPAYQQGQNQLYNELNLGRREEYDVLDKRRGRDPEMGGKPQRRKNPQEGLYNELQKDKMAEAYSEIGMKGERRRGKGHDGLYQGLSTATKDTYDALHMQALPPREGRGSLLTCGDVEENPGPRISKPHLRSISIQCYLCLLLNSHFLTEAGIHVFILGCFSAGLPKTEANWVNVISDLKKIEDLIQSMHIDATLYTESDVHPSCKVTAMKCFLLELQVISLESGDASIHDTVENLIILANNSLSSNGNVTESGCKECEELEEKNIKEFLQSFVHIVQMFINTS

SEQ ID NO: 15 - protein, 618 aa, synthetic construct
MALPVTALLLPLALLLHAARPEVQLQASGGGLAQPGGSLRLSCAASGRTFSTYFMAWFRQPPGKGLEYVGGIRWSDGVPHYADSVKGRFTISRDNAKNTVYLQMNSLRAEDTAVYFCASRGIADGSDFGSYGQGTQVTVSSIEVMYPPPYLDNEKSNGTIIHVKGKHLCPSPLFPGPSKPFWVLVVVGGVLACYSLLVTVAFIIFWVRRKRKEKQSETSPKEFLTIYEDVKDLKTRRNHEQEQTFPGGGSTIYSMIQSQSSAPTSQEPAYTLYSLIQPSRKSGSRKRNHSPSFNSTIYEVIGKSQPKAQNPARLSRKELENFDVYSRVKFSRSADAPAYQQGQNQLYNELNLGRREEYDVLDKRRGRDPEMGGKPQRRKNPQEGLYNELQKDKMAEAYSEIGMKGERRRGKGHDGLYQGLSTATKDTYDALHMQALPPREGRGSLLTCGDVEENPGPRISKPHLRSISIQCYLCLLLNSHFLTEAGIHVFILGCFSAGLPKTEANWVNVISDLKKIEDLIQSMHIDATLYTESDVHPSCKVTAMKCFLLELQVISLESGDASIHDTVENLIILANNSLSSNGNVTESGCKECEELEEKNIKEFLQSFVHIVQMFINTS

SEQ ID NO: 16 - DNA, 360 bp, synthetic construct
  source 1..360: mol_type = other DNA
gaagtccaactccaggcttccggtggcggtctggcacagcctggagggtccctgcggctctcctgcgcagcaagtggcaggactttcagtacctactttatggcctggttcagacagccacctggcaaaggcctcgaatacgtcggagggattaggtggtctgacggtgtccctcactacgctgacagtgtgaagggtcggttcaccattagcagagacaacgctaagaatacagtgtacctgcaaatgaactcactgagagctgaggatactgctgtgtacttctgcgcatctcgcggaatcgctgacgggtcagactttggctcctatggacagggcacccaggtgactgtgagttcc

SEQ ID NO: 17 - DNA, 321 bp, synthetic construct
  source 1..321: mol_type = other DNA
attgaagttatgtatcctcctccttacctagacaatgagaagagcaatggaaccattatccatgtgaaagggaaacacctttgtccaagtcccctatttcccggaccttctaagcccttttgggtgctggtggtggttggtggagtcctggcttgctatagcttgctagtaacagtggcctttattattttctgggtgaggagtaagaggagcaggctcctgcacagtgactacatgaacatgactccccgccgccccgggcccacccgcaagcattaccagccctatgccccaccacgcgacttcgcagcctatcgctcc

SEQ ID NO: 18 - DNA, 339 bp, synthetic construct
  source 1..339: mol_type = other DNA
agagtgaagttcagcaggagcgcagacgcccccgcgtaccagcagggccagaaccagctctataacgagctcaatctaggacgaagagaggagtacgatgttttggacaagagacgtggccgggaccctgagatggggggaaagccgcagagaaggaagaaccctcaggaaggcctgtacaatgaactgcagaaagataagatggcggaggcctacagtgagattgggatgaaaggcgagcgccggaggggcaaggggcacgatggcctttaccagggtctcagtacagccaccaaggacacctacgacgcccttcacatgcaggccctgccccctcgc

SEQ ID NO: 19 - DNA, 54 bp, synthetic construct
  source 1..54: mol_type = other DNA
gagggcagaggaagtcttctaacatgcggtgacgtggaggagaatcccggccct

SEQ ID NO: 20 - DNA, 486 bp, synthetic construct
  source 1..486: mol_type = other DNA
agaatttcgaaaccacatttgagaagtatttccatccagtgctacttgtgtttacttctaaacagtcattttctaactgaagctggcattcatgtcttcattttgggctgtttcagtgcagggcttcctaaaacagaagccaactgggtgaatgtaataagtgatttgaaaaaaattgaagatcttattcaatctatgcatattgatgctactttatatacggaaagtgatgttcaccccagttgcaaagtaacagcaatgaagtgctttctcttggagttacaagttatttcacttgagtccggagatgcaagtattcatgatacagtagaaaatctgatcatcctagcaaacaacagtttgtcttctaatgggaatgtaacagaatctggatgcaaagaatgtgaggaactggaggaaaaaaatattaaagaatttttgcagagttttgtacatattgtccaaatgttcatcaacacttcttga

SEQ ID NO: 21 - DNA, 1020 bp, synthetic construct
  source 1..1020: mol_type = other DNA
gaagtccaactccaggcttccggtggcggtctggcacagcctggagggtccctgcggctctcctgcgcagcaagtggcaggactttcagtacctactttatggcctggttcagacagccacctggcaaaggcctcgaatacgtcggagggattaggtggtctgacggtgtccctcactacgctgacagtgtgaagggtcggttcaccattagcagagacaacgctaagaatacagtgtacctgcaaatgaactcactgagagctgaggatactgctgtgtacttctgcgcatctcgcggaatcgctgacgggtcagactttggctcctatggacagggcacccaggtgactgtgagttccattgaagttatgtatcctcctccttacctagacaatgagaagagcaatggaaccattatccatgtgaaagggaaacacctttgtccaagtcccctatttcccggaccttctaagcccttttgggtgctggtggtggttggtggagtcctggcttgctatagcttgctagtaacagtggcctttattattttctgggtgaggagtaagaggagcaggctcctgcacagtgactacatgaacatgactccccgccgccccgggcccacccgcaagcattaccagccctatgccccaccacgcgacttcgcagcctatcgctccagagtgaagttcagcaggagcgcagacgcccccgcgtaccagcagggccagaaccagctctataacgagctcaatctaggacgaagagaggagtacgatgttttggacaagagacgtggccgggaccctgagatggggggaaagccgcagagaaggaagaaccctcaggaaggcctgtacaatgaactgcagaaagataagatggcggaggcctacagtgagattgggatgaaaggcgagcgccggaggggcaaggggcacgatggcctttaccagggtctcagtacagccaccaaggacacctacgacgcccttcacatgcaggccctgccccctcgc

SEQ ID NO: 22 - DNA, 1083 bp, synthetic construct
  source 1..1083: mol_type = other DNA
atggccttaccagtgaccgccttgctcctgccgctggccttgctgctccacgccgccaggccggaagtccaactccaggcttccggtggcggtctggcacagcctggagggtccctgcggctctcctgcgcagcaagtggcaggactttcagtacctactttatggcctggttcagacagccacctggcaaaggcctcgaatacgtcggagggattaggtggtctgacggtgtccctcactacgctgacagtgtgaagggtcggttcaccattagcagagacaacgctaagaatacagtgtacctgcaaatgaactcactgagagctgaggatactgctgtgtacttctgcgcatctcgcggaatcgctgacgggtcagactttggctcctatggacagggcacccaggtgactgtgagttccattgaagttatgtatcctcctccttacctagacaatgagaagagcaatggaaccattatccatgtgaaagggaaacacctttgtccaagtcccctatttcccggaccttctaagcccttttgggtgctggtggtggttggtggagtcctggcttgctatagcttgctagtaacagtggcctttattattttctgggtgaggagtaagaggagcaggctcctgcacagtgactacatgaacatgactccccgccgccccgggcccacccgcaagcattaccagccctatgccccaccacgcgacttcgcagcctatcgctccagagtgaagttcagcaggagcgcagacgcccccgcgtaccagcagggccagaaccagctctataacgagctcaatctaggacgaagagaggagtacgatgttttggacaagagacgtggccgggaccctgagatggggggaaagccgcagagaaggaagaaccctcaggaaggcctgtacaatgaactgcagaaagataagatggcggaggcctacagtgagattgggatgaaaggcgagcgccggaggggcaaggggcacgatggcctttaccagggtctcagtacagccaccaaggacacctacgacgcccttcacatgcaggccctgccccctcgc

SEQ ID NO: 23 - DNA, 1623 bp, synthetic construct
  source 1..1623: mol_type = other DNA
atggccttaccagtgaccgccttgctcctgccgctggccttgctgctccacgccgccaggccggaagtccaactccaggcttccggtggcggtctggcacagcctggagggtccctgcggctctcctgcgcagcaagtggcaggactttcagtacctactttatggcctggttcagacagccacctggcaaaggcctcgaatacgtcggagggattaggtggtctgacggtgtccctcactacgctgacagtgtgaagggtcggttcaccattagcagagacaacgctaagaatacagtgtacctgcaaatgaactcactgagagctgaggatactgctgtgtacttctgcgcatctcgcggaatcgctgacgggtcagactttggctcctatggacagggcacccaggtgactgtgagttccattgaagttatgtatcctcctccttacctagacaatgagaagagcaatggaaccattatccatgtgaaagggaaacacctttgtccaagtcccctatttcccggaccttctaagcccttttgggtgctggtggtggttggtggagtcctggcttgctatagcttgctagtaacagtggcctttattattttctgggtgaggagtaagaggagcaggctcctgcacagtgactacatgaacatgactccccgccgccccgggcccacccgcaagcattaccagccctatgccccaccacgcgacttcgcagcctatcgctccagagtgaagttcagcaggagcgcagacgcccccgcgtaccagcagggccagaaccagctctataacgagctcaatctaggacgaagagaggagtacgatgttttggacaagagacgtggccgggaccctgagatggggggaaagccgcagagaaggaagaaccctcaggaaggcctgtacaatgaactgcagaaagataagatggcggaggcctacagtgagattgggatgaaaggcgagcgccggaggggcaaggggcacgatggcctttaccagggtctcagtacagccaccaaggacacctacgacgcccttcacatgcaggccctgccccctcgcgagggcagaggaagtcttctaacatgcggtgacgtggaggagaatcccggccctagaatttcgaaaccacatttgagaagtatttccatccagtgctacttgtgtttacttctaaacagtcattttctaactgaagctggcattcatgtcttcattttgggctgtttcagtgcagggcttcctaaaacagaagccaactgggtgaatgtaataagtgatttgaaaaaaattgaagatcttattcaatctatgcatattgatgctactttatatacggaaagtgatgttcaccccagttgcaaagtaacagcaatgaagtgctttctcttggagttacaagttatttcacttgagtccggagatgcaagtattcatgatacagtagaaaatctgatcatcctagcaaacaacagtttgtcttctaatgggaatgtaacagaatctggatgcaaagaatgtgaggaactggaggaaaaaaatattaaagaatttttgcagagttttgtacatattgtccaaatgttcatcaacacttcttga

SEQ ID NO: 24 - protein, 242 aa, synthetic construct
DIQMTQTTSSLSASLGDRVTISCRASQDISKYLNWYQQKPDGTVKLLIYHTSRLHSGVPSRFSGSGSGTDYSLTISNLEQEDIATYFCQQGNTLPYTFGGGTKLEITGGGGSGGGGSGGGGSEVKLQESGPGLVAPSQSLSVTCTVSGVSLPDYGVSWIRQPPRKGLEWLGVIWGSETTYYNSALKSRLTIIKDNSKSQVFLKMNSLQTDDTAIYYCAKHYYYGGSYAMDYWGQGTSVTVSS